European Patent Application EP 4 471 060 A1, published December 4, 2024. Title: ANTI-INTERLEUKIN-11 ANTIBODY AND USE THEREOF. Applicant: MABWELL (SHANGHAI) BIOSCIENCE CO., LTD. The sequence listing filed with the application follows.

SEQUENCE LISTING (162 sequences)

SEQ ID NO: 1 - protein, 119 aa, synthetic construct
  REGION 1..119: note = VH
EVQLVQSGAEVKKPGASVKISCKASGYTFTDYNMDWVKQAPGQRLEWIGDINPHNGGPIYNQKFTGRATLTVDKSASTAYMELSSLRSEDTAVYYCARGELGHWYFDVWGQGTTVTVSS

SEQ ID NO: 2 - protein, 111 aa, synthetic construct
  REGION 1..111: note = VL
DIVLTQSPASLALSPGERATLSCRASKSVSTSGYSYIHWYQQKPGQAPRLLIYLASNLDSGVPARFSGSGSGTDFTLTISSLEEEDFATYYCQHSRDLPPTFGQGTKLEIK

SEQ ID NO: 3 - protein, 324 aa, synthetic construct
  REGION 1..324: note = CH
AKTTPPSVYPLAPGSAAQTNSMVTLGCLVKGYFPEPVTVTWNSGSLSSGVHTFPAVLQSDLYTLSSSVTVPSSTWPSETVTCNVAHPASSTKVDKKIVPRDCGCKPCICTVPEVSSVFIFPPKPKDVLTITLTPKVTCVVVDISKDDPEVQFSWFVDDVEVHTAQTQPREEQFNSTFRSVSELPIMHQDWLNGKEFKCRVNSAAFPAPIEKTISKTKGRPKAPQVYTIPPPKEQMAKDKVSLTCMITDFFPEDITVEWQWNGQPAENYKNTQPIMDTDGSYFVYSKLNVQKSNWEAGNTFTCSVLHEGLHNHHTEKSLSHSPGK

SEQ ID NO: 4 - protein, 107 aa, synthetic construct
  REGION 1..107: note = CL
RTVAAPTVSIFPPSSEQLTSGGASVVCFLNNFYPKDINVKWKIDGSERQNGVLNSWTDQDSKDSTYSMSSTLTLTKDEYERHNSYTCEATHKTSTSPIVKSFNRNEC

SEQ ID NO: 5 - protein, 117 aa, synthetic construct
  REGION 1..117: note = VH
QVQLQQPGAELVKPGASVKMSCKASGYKFITYNMDWVKQTPGQGLEWIGTIYPGNGDTSYNQKFKGKATLTADKSSSTAYMQLSSLTSEDSAVYYCARGDLYALDYWGQGTSVTVSS

SEQ ID NO: 6 - protein, 108 aa, synthetic construct
  REGION 1..108: note = VL
SIVMTQTPKFLLVSAGDRVTITCKASQSVSNDVAWYQQKPGQSPKLLIYSASNRYTGVPDRFTGSGYGTDFTFTINTVQAEDLAVYFCQHDYSSPYTFGGGTKLEIKR

SEQ ID NO: 7 - protein, 120 aa, synthetic construct
  REGION 1..120: note = VH
DVQLVESGGGLVQPGGSRKLSCAASGFTFSSFGMHWVRQSPERGLEWVAYITSGSNTIYYADTVKGRFTISRDNPENTLFLQMTSLRSEDTAMYYCAREYYSYDEGFAYWGQGTLVTVSA

SEQ ID NO: 8 - protein, 109 aa, synthetic construct
  REGION 1..109: note = VL
EIVLTQSPTTMAASPGEKITITCSVSSSISSNYLHWYQQKPGFSPKLLIYRTSNLASGVPARFSGSGSGTSHSLTIDTMEAEDVATYYCQQGVDVPFTFGSGTKLEIKR

SEQ ID NO: 9 - protein, 117 aa, synthetic construct
  REGION 1..117: note = VH
EVQLVQSGAEVKKPGASVKVSCKASGYTFTTYNMDWVRQAPGQGLEWMGTIYPGNGDTSYNQKFKGRVTMTRDTSTSTVYMELSSLRSEDTAVYYCARGDLYALDYWGQGTLVTVSS

SEQ ID NO: 10 - protein, 107 aa, synthetic construct
  REGION 1..107: note = VL
DIQMTQSPSSLSASVGDRVTITCKASQSVSNDVAWYQQKPGKAPKLLIYSASNRYTGVPSRFSGSGSGTDFTFTISSLQPEDIATYYCQHDYSSPYTFGQGTKLEIK

SEQ ID NO: 11 - protein, 120 aa, synthetic construct
  REGION 1..120: note = VH
EVQLVESGGGLVQPGGSLRLSCAASGFTFSSFGMHWVRQAPGKGLEWVAYITSGSNTIYYADTVKGRFTISRDNAKNSLYLQMNSLRAEDTAVYYCAREYYSYDEGFAYWGQGTLVTVSS

SEQ ID NO: 12 - protein, 108 aa, synthetic construct
  REGION 1..108: note = VL
EIVLTQSPATLSLSPGERATLSCSVSSSISSNYLHWYQQKPGQAPRLLIYRTSNLASGIPARFSGSGSGTDFTLTISSLEPEDFAVYYCQQGVDVPFTFGQGTKLEIK

SEQ ID NO: 13 - protein, 330 aa, synthetic construct [sequence omitted]

SEQ ID NO: 14 - protein, 107 aa, synthetic construct [sequence omitted]

SEQ ID NO: 15 - protein, 120 aa, synthetic construct
  REGION 1..120: note = VH
EVQLVESGGGLVQPGGSLRLSCAASGFTFSSFGMHWVRQAPGKGLEWVAYITPGSNTIYYADTVKGRFTISRDNAKNSLYLQMNSLRAEDTAVYYCAREYYSYDEGFAYWGQGTLVTVSS

SEQ ID NO: 16 - protein, 120 aa, synthetic construct
  REGION 1..120: note = VH
EVQLVESGGGLVQPGGSLRLSCAASGFTFSSFGMHWVRQAPGKGLEWVAYITAGSNTIYYADTVKGRFTISRDNAKNSLYLQMNSLRAEDTAVYYCAREYYSYDEGFAYWGQGTLVTVSS

SEQ ID NO: 17 - protein, 120 aa, synthetic construct
  REGION 1..120: note = VH
EVQLVESGGGLVQPGGSLRLSCAASGFTFSSFGMHWVRQAPGKGLEWVAYITPGSNTTYYADTVKGRFTISRDNAKNSLYLQMNSLRAEDTAVYYCAREYYSYDEGFAYWGQGTLVTVSS

SEQ ID NO: 18 - protein, 120 aa, synthetic construct
  REGION 1..120: note = VH
EVQLVESGGGLVQPGGSLRLSCAASGFTFSSFGMHWVRQAPGKGLEWVAYITSGANTIYYADTVKGRFTISRDNAKNSLYLQMNSLRAEDTAVYYCAREYYSYDEGFAYWGQGTLVTVSS

SEQ ID NO: 19 - protein, 120 aa, synthetic construct
  REGION 1..120: note = VH
EVQLVESGGGLVQPGGSLRLSCAASGFTFSSFGMSWVRQAPGKGLEWVAYITPGSNTIYYADTVKGRFTISRDNAKNSLYLQMNSLRAEDTAVYYCAREYYSYDEGFAYWGQGTLVTVSS

SEQ ID NO: 20 - protein, 120 aa, synthetic construct
  REGION 1..120: note = VH
EVQLVESGGGLVQPGGSLRLSCAASGFTFSSFGMHWVRQAPGKGLEWVAYITPGSSTIYYADTVKGRFTISRDNAKNSLYLQMNSLRAEDTAVYYCAREYYSYDEGFAYWGQGTLVTVSS

SEQ ID NO: 21 - protein, 120 aa, synthetic construct
  REGION 1..120: note = VH
EVQLVESGGGLVQPGGSLRLSCAASGFTFSSYGMHWVRQAPGKGLEWVAYITPGSNTIYYADTVKGRFTISRDNAKNSLYLQMNSLRAEDTAVYYCAREYYSYDEGFAYWGQGTLVTVSS

SEQ ID NO: 22 - protein, 120 aa, synthetic construct
  REGION 1..120: note = VH
EVQLVESGGGLVQPGGSLRLSCAASGFTFSSFGMHWVRQAPGKGLEWVASITPGSNTIYYADTVKGRFTISRDNAKNSLYLQMNSLRAEDTAVYYCAREYYSYDEGFAYWGQGTLVTVSS

SEQ ID NO: 23 - protein, 120 aa, synthetic construct
  REGION 1..120: note = VH
EVQLVESGGGLVQPGGSLRLSCAASGFTFSSFGMHWVRQAPGKGLEWVAYITPGSNTIYYADTVKGRFTISRDNAKNSLYLQMNSLRAEDTAVYYCAREYSSYDEGFAYWGQGTLVTVSS

SEQ ID NO: 24 - protein, 120 aa, synthetic construct
  REGION 1..120: note = VH
EVQLVESGGGLVQPGGSLRLSCAASGFTFSSFGMHWVRQAPGKGLEWVSYITPGSNTIYYADTVKGRFTISRDNAKNSLYLQMNSLRAEDTAVYYCAREYYSYDEGFAYWGQGTLVTVSS

SEQ ID NO: 25 - protein, 120 aa, synthetic construct
  REGION 1..120: note = VH
EVQLVESGGGLVQPGGSLRLSCAASGFTFSSFGMHWVRQAPGKGLEYVAYITPGSNTIYYADTVKGRFTISRDNAKNSLYLQMNSLRAEDTAVYYCAREYYSYDEGFAYWGQGTLVTVSS

SEQ ID NO: 26 - protein, 120 aa, synthetic construct
  REGION 1..120: note = VH
EVQLVESGGGLVQPGGSLRLSCAASGFTFSSFGMHWVRQAPGKGLEWVAVITPGSNTIYYADTVKGRFTISRDNAKNSLYLQMNSLRAEDTAVYYCAREYYSYDEGFAYWGQGTLVTVSS

SEQ ID NO: 27 - protein, 120 aa, synthetic construct
  REGION 1..120: note = VH
EVQLVESGGGLVQPGGSLRLSCAASGFTFSSFGMHWVRQAPGKGLEWVSVITPGSNTIYYADTVKGRFTISRDNAKNSLYLQMNSLRAEDTAVYYCAREYYSYDEGFAYWGQGTLVTVSS

SEQ ID NO: 28 - protein, 120 aa, synthetic construct
  REGION 1..120: note = VH
EVQLVESGGGLVQPGGSLRLSCAASGFTFSSFGMHWVRQAPGKGLEWIGYITPGSNTIYYADTVKGRFTISRDNAKNSLYLQMNSLRAEDTAVYYCAREYYSYDEGFAYWGQGTLVTVSS

SEQ ID NO: 29 - protein, 120 aa, synthetic construct
  REGION 1..120: note = VH
EVQLVESGGGLVQPGGSLRLSCAASGFTFSSFGMHWVRQAPGKGLEWMGYITPGSNTIYYADTVKGRFTISRDNAKNSLYLQMNSLRAEDTAVYYCAREYYSYDEGFAYWGQGTLVTVSS

SEQ ID NO: 30 - protein, 120 aa, synthetic construct
  REGION 1..120: note = VH
EVQLVESGGGLVQPGGSLRLSCAASGFTFSSFGMHWVRQAPGKGLEWVAYITPGSNTIYYADTVKGRFTISRDNAKNSLYLQMNSLRAEDTAVYYCAREYYSSDEGFAYWGQGTLVTVSS

SEQ ID NO: 31 - protein, 120 aa, synthetic construct
  REGION 1..120: note = VH
EVQLVESGGGLVQPGGSLRLSCAASGFTFSSFGMHWVRQAPGKGLEWVAYITPGSNTIYYADTVKGRFTISRDNAKNSLYLQMNSLRAEDTAVYYCAREYYSYDEGPAYWGQGTLVTVSS

SEQ ID NO: 32 - protein, 120 aa, synthetic construct
  REGION 1..120: note = VH
EVQLVESGGGLVQPGGSLRLSCAASGFTFSSFGMHWVRQAPGKGLEWVAYITPGSNTIYYADTVKGRFTISRDNAKNSLYLQMNSLRAEDTAVYYCAREYYSYDEGGAYWGQGTLVTVSS

SEQ ID NO: 33 - protein, 120 aa, synthetic construct
  REGION 1..120: note = VH
EVQLVESGGGLVQPGGSLRLSCAASGFTFSSFGMHWVRQAPGKGLEWVAYITPGSNTIYYADTVKGRFTISRDNAKNSLYLQMNSLRAEDTAVYYCAREYYSYDEGFASWGQGTLVTVSS

SEQ ID NO: 34 - protein, 108 aa, synthetic construct
  REGION 1..108: note = VL
EIVLTQSPATLSLSPGERATLSCSVSSSIPSNYLHWYQQKPGQAPRLLIYRTSNLASGIPARFSGSGSGTDFTLTISSLEPEDFAVYYCQQGVDVPFTFGQGTKLEIK

SEQ ID NO: 35 - protein, 108 aa, synthetic construct
  REGION 1..108: note = VL
EIVLTQSPATLSLSPGERATLSCSVSSSISSKYLHWYQQKPGQAPRLLIYRTSNLASGIPARFSGSGSGTDFTLTISSLEPEDFAVYYCQQGVDVPFTFGQGTKLEIK

SEQ ID NO: 36 - protein, 108 aa, synthetic construct
  REGION 1..108: note = VL
EIVLTQSPATLSLSPGERATLSCSVSSLISSNYLHWYQQKPGQAPRLLIYRTSNLASGIPARFSGSGSGTDFTLTISSLEPEDFAVYYCQQGVDVPFTFGQGTKLEIK

SEQ ID NO: 37 - protein, 108 aa, synthetic construct
  REGION 1..108: note = VL
EIVLTQSPATLSLSPGERATLSCSVSDLISSNYLHWYQQKPGQAPRLLIYRTSNLASGIPARFSGSGSGTDFTLTISSLEPEDFAVYYCQQGVDVPFTFGQGTKLEIK

SEQ ID NO: 38 - protein, 108 aa, synthetic construct
  REGION 1..108: note = VL
EIVLTQSPATLSLSPGERATLSCSVSELLSTNYLHWYQQKPGQAPRLLIYRTSNLASGIPARFSGSGSGTDFTLTISSLEPEDFAVYYCQQGVDVPFTFGQGTKLEIK

SEQ ID NO: 39 - protein, 108 aa, synthetic construct
  REGION 1..108: note = VL
EIVLTQSPATLSLSPGERATLSCSVSSLIPSKYLHWYQQKPGQAPRLLIYRTSNLASGIPARFSGSGSGTDFTLTISSLEPEDFAVYYCQQGVDVPFTFGQGTKLEIK

SEQ ID NO: 40 - protein, 108 aa, synthetic construct
  REGION 1..108: note = VL
EIVLTQSPATLSLSPGERATLSCSVSDLIPSQYLHWYQQKPGQAPRLLIYRTSNLASGIPARFSGSGSGTDFTLTISSLEPEDFAVYYCQQGVDVPFTFGQGTKLEIK

SEQ ID NO: 41 - protein, 108 aa, synthetic construct
  REGION 1..108: note = VL
EIVLTQSPATLSLSPGERATLSCSVSDLIPSQYLSWYQQKPGQAPRLLIYRTSNLASGIPARFSGSGSGTDFTLTISSLEPEDFAVYYCQQGVDVPFTFGQGTKLEIK

SEQ ID NO: 42 - protein, 108 aa, synthetic construct
  REGION 1..108: note = VL
EIVLTQSPATLSLSPGERATLSCSVSDLIPSQYLAWYQQKPGQAPRLLIYRTSNLASGIPARFSGSGSGTDFTLTISSLEPEDFAVYYCQQGVDVPFTFGQGTKLEIK

SEQ ID NO: 43 - protein, 108 aa, synthetic construct
  REGION 1..108: note = VL
EIVLTQSPATLSLSPGERATLSCSVSDLIPSQYLHWYQQKPGQAPRLLIYRASNLASGIPARFSGSGSGTDFTLTISSLEPEDFAVYYCQQGVDVPFTFGQGTKLEIK

SEQ ID NO: 44 - protein, 108 aa, synthetic construct
  REGION 1..108: note = VL
EIVLTQSPATLSLSPGERATLSCSVSDLIPSQYLHWYQQKPGQAPRLLIYDASNLASGIPARFSGSGSGTDFTLTISSLEPEDFAVYYCQQGVDVPFTFGQGTKLEIK

SEQ ID NO: 45 - protein, 108 aa, synthetic construct
  REGION 1..108: note = VL
EIVLTQSPATLSLSPGERATLSCSVSDLIPSQYLHWYQQKPGQAPRLLIYGASNLASGIPARFSGSGSGTDFTLTISSLEPEDFAVYYCQQGVDVPFTFGQGTKLEIK

SEQ ID NO: 46 - protein, 108 aa, synthetic construct
  REGION 1..108: note = VL
EIVLTQSPATLSLSPGERATLSCSVSDLIPSQYLHWYQQKPGQAPRLLIYRTSNRASGIPARFSGSGSGTDFTLTISSLEPEDFAVYYCQQGVDVPFTFGQGTKLEIK

SEQ ID NO: 47 - protein, 115 aa, synthetic construct
  REGION 1..115: note = VH
QVQLVQSGAEVKKPGSSVKVSCKASGFTFTTYYISWVRQAPGQGLEYLGYINMGSGGTNYNEKFKGRVTITADKSTSTAYMELSSLRSEDTAVYYCAIIGYFDYWGQGTMVTVSS

SEQ ID NO: 48 - protein, 112 aa, synthetic construct
  REGION 1..112: note = VL
DVVMTQSPLSLPVTLGQPASISCRSSQSLLDSDGGTYLYWFQQRPGQSPRRLIYLVSTLGSGVPDRFSGSGSGTDFTLKISRVEAEDVGVYYCMQLTHWPYTFGQGTKLEIK

SEQ ID NO: 49 - protein, 117 aa, synthetic construct
  REGION 1..117: note = VH
EVQLVQSGAEVKKPGASVKVSCKASGYTFTTYNMDWVRQAPGQGLEWMGTIYPGNGDTSYNQKFKGRVTMTRDTSTSTVYMELSSLRSEDTAVYYCARGDLHFLDYWGQGTLVTVSS

SEQ ID NO: 50 - protein, 117 aa, synthetic construct
  REGION 1..117: note = VH
EVQLVQSGAEVKKPGASVKVSCKASGYTFTTYNMDWVRQAPGQGLEWMGTIYPGNGDTSYNQKFKGRVTMTRDTSTSTVYMELSSLRSEDTAVYYCARGDLHYLDYWGQGTLVTVSS

SEQ ID NO: 51 - protein, 117 aa, synthetic construct
  REGION 1..117: note = VH
EVQLVQSGAEVKKPGASVKVSCKASGYTFTTYDMDWVRQAPGQGLEWMGTIYPGNGDTSYNQKFKGRVTMTRDTSTSTVYMELSSLRSEDTAVYYCARGDLYALDYWGQGTLVTVSS

SEQ ID NO: 52 - protein, 117 aa, synthetic construct
  REGION 1..117: note = VH
EVQLVQSGAEVKKPGASVKVSCKASGYTFTTYNIDWVRQAPGQGLEWMGTIYPGNGDTSYNQKFKGRVTMTRDTSTSTVYMELSSLRSEDTAVYYCARGDLYALDYWGQGTLVTVSS

SEQ ID NO: 53 - protein, 117 aa, synthetic construct
  REGION 1..117: note = VH
EVQLVQSGAEVKKPGASVKVSCKASGYTFITYNMDWVRQAPGQGLEWMGTIYPGNGDTSYNQKFKGRVTMTRDTSTSTAYMELSSLRSEDTAVYYCARADLHFLDYWGQGTLVTVSS

SEQ ID NO: 54 - protein, 117 aa, synthetic construct
  REGION 1..117: note = VH
EVQLVQSGAEVKKPGASVKVSCKASGYTFNHYDMDWVRQAPGQGLEWMGTIYPGNGDTSYNQKFKGRVTMTRDTSTSTVYMELSSLRSEDTAVYYCARGDLYALDYWGQGTLVTVSS

SEQ ID NO: 55 - protein, 117 aa, synthetic construct
  REGION 1..117: note = VH
EVQLVQSGAEVKKPGASVKVSCKASGYTFTTYDIDWVRQAPGQGLEWMGTIYPGNGDTSYNQKFKGRVTMTRDTSTSTVYMELSSLRSEDTAVYYCARGDLYALDYWGQGTLVTVSS

SEQ ID NO: 56 - protein, 117 aa, synthetic construct
  REGION 1..117: note = VH
EVQLVQSGAEVKKPGASVKVSCKASGYTFTTYDMHWVRQAPGQGLEWMGTIYPGNGDTSYNQKFKGRVTMTRDTSTSTVYMELSSLRSEDTAVYYCARGDLYALDYWGQGTLVTVSS

SEQ ID NO: 57 - protein, 117 aa, synthetic construct
  REGION 1..117: note = VH
EVQLVQSGAEVKKPGASVKVSCKASGYTFTTYDMSWVRQAPGQGLEWMGTIYPGNGDTSYNQKFKGRVTMTRDTSTSTVYMELSSLRSEDTAVYYCARGDLYALDYWGQGTLVTVSS

SEQ ID NO: 58 - protein, 117 aa, synthetic construct
  REGION 1..117: note = VH
EVQLVQSGAEVKKPGASVKVSCKASGYTFNHYNMDWVRQAPGQGLEWMGTIYPGNGDTSYNQKFKGRVTMTRDTSTSTVYMELSSLRSEDTAVYYCARGDLYALDYWGQGTLVTVSS

SEQ ID NO: 59 - protein, 117 aa, synthetic construct
  REGION 1..117: note = VH
EVQLVQSGAEVKKPGASVKVSCKASGYTFTHYNMDWVRQAPGQGLEWMGTIYPGNGDTSYNQKFKGRVTMTRDTSTSTVYMELSSLRSEDTAVYYCARGDLYALDYWGQGTLVTVSS

SEQ ID NO: 60 - protein, 117 aa, synthetic construct
  REGION 1..117: note = VH
EVQLVQSGAEVKKPGASVKVSCKASGYTFTHYDMDWVRQAPGQGLEWMGTIYPGNGDTSYNQKFKGRVTMTRDTSTSTVYMELSSLRSEDTAVYYCARGDLYALDYWGQGTLVTVSS

SEQ ID NO: 61 - protein, 117 aa, synthetic construct
  REGION 1..117: note = VH
EVQLVQSGAEVKKPGASVKVSCKASGYTFTHYEMDWVRQAPGQGLEWMGTIYPGNGDTSYNQKFKGRVTMTRDTSTSTVYMELSSLRSEDTAVYYCARGDLYALDYWGQGTLVTVSS

SEQ ID NO: 62 - protein, 117 aa, synthetic construct
  REGION 1..117: note = VH
EVQLVQSGAEVKKPGASVKVSCKASGYTFTHYQMDWVRQAPGQGLEWMGTIYPGNGDTSYNQKFKGRVTMTRDTSTSTVYMELSSLRSEDTAVYYCARGDLYALDYWGQGTLVTVSS

SEQ ID NO: 63 - protein, 117 aa, synthetic construct
  REGION 1..117: note = VH
EVQLVQSGAEVKKPGASVKVSCKASGYTFTHYSMDWVRQAPGQGLEWMGTIYPGNGDTSYNQKFKGRVTMTRDTSTSTVYMELSSLRSEDTAVYYCARGDLYALDYWGQGTLVTVSS

SEQ ID NO: 64 - protein, 117 aa, synthetic construct
  REGION 1..117: note = VH
EVQLVQSGAEVKKPGASVKVSCKASGYTFTHYDMDWVRQAPGQGLEWMGTIYPGNADTSYNQKFKGRVTMTRDTSTSTVYMELSSLRSEDTAVYYCARGDLYALDYWGQGTLVTVSS

SEQ ID NO: 65 - protein, 117 aa, synthetic construct
  REGION 1..117: note = VH
EVQLVQSGAEVKKPGASVKVSCKASGYTFTHYDMDWVRQAPGQGLEWMGTIYPGEGDTSYNQKFKGRVTMTRDTSTSTVYMELSSLRSEDTAVYYCARGDLYALDYWGQGTLVTVSS

SEQ ID NO: 66 - protein, 117 aa, synthetic construct
  REGION 1..117: note = VH
EVQLVQSGAEVKKPGASVKVSCKASGYTFTHYNMDWVRQAPGQGLEWMGTIYPGEGDTSYNQKFKGRVTMTRDTSTSTVYMELSSLRSEDTAVYYCARGDLYALDYWGQGTLVTVSS

SEQ ID NO: 67 - protein, 117 aa, synthetic construct
  REGION 1..117: note = VH
EVQLVQSGAEVKKPGASVKVSCKASGYTFTHYNMDWVRQAPGQGLEWMGTIYPGNADTSYNQKFKGRVTMTRDTSTSTVYMELSSLRSEDTAVYYCARGDLYALDYWGQGTLVTVSS

SEQ ID NO: 68 - protein, 117 aa, synthetic construct
  REGION 1..117: note = VH
EVQLVQSGAEVKKPGASVKVSCKASGYTFTHYNMDWVRQAPGQGLEWMGTIYPGQGDTSYNQKFKGRVTMTRDTSTSTVYMELSSLRSEDTAVYYCARGDLYALDYWGQGTLVTVSS

SEQ ID NO: 69 - protein, 107 aa, synthetic construct
  REGION 1..107: note = VL
DIQMTQSPSSLSASVGDRVTITCKASKSVSNDVAWYQQKPGKAPKLLIYSASNRYTGVPSRFSGSGSGTDFTFTISSLQPEDIATYYCQHDYSSPYTFGQGTKLEIK

SEQ ID NO: 70 - protein, 107 aa, synthetic construct
  REGION 1..107: note = VL
DIQMTQSPSSLSASVGDRVTITCKASYSVSNDVAWYQQKPGKAPKLLIYSASNRYTGVPSRFSGSGSGTDFTFTISSLQPEDIATYYCQHDYSSPYTFGQGTKLEIK

SEQ ID NO: 71 - protein, 107 aa, synthetic construct
  REGION 1..107: note = VL
DIQMTQSPSSLSASVGDRVTITCKASHSVSNDVAWYQQKPGKAPKLLIYSASNRYTGVPSRFSGSGSGTDFTFTISSLQPEDIATYYCQHDYSSPYTFGQGTKLEIK

SEQ ID NO: 72 - protein, 107 aa, synthetic construct
  REGION 1..107: note = VL
DIQMTQSPSSLSASVGDRVTITCKASQFVSNDVAWYQQKPGKAPKLLIYSASNRYTGVPSRFSGSGSGTDFTFTISSLQPEDIATYYCQHDYSSPYTFGQGTKLEIK

SEQ ID NO: 73 - protein, 107 aa, synthetic construct
  REGION 1..107: note = VL
DIQMTQSPSSLSASVGDRVTITCKASQSVSNDIAWYQQKPGKAPKLLIYSASNRYTGVPSRFSGSGSGTDFTFTISSLQPEDIATYYCQHDYSSPYTFGQGTKLEIK

SEQ ID NO: 74 - protein, 107 aa, synthetic construct
  REGION 1..107: note = VL
DIQMTQSPSSLSASVGDRVTITCKASQSVFHDVAWYQQKPGKAPKLLIYSASNRYTGVPSRFSGSGSGTDFTFTISSLQPEDIATYYCQHDYSSPYTFGQGTKLEIK

SEQ ID NO: 75 - protein, 107 aa, synthetic construct
  REGION 1..107: note = VL
DIQMTQSPSSLSASVGDRVTITCKASQSVFRDVAWYQQKPGKAPKLLIYSASNRYTGVPSRFSGSGSGTDFTFTISSLQPEDIATYYCQHDYSSPYTFGQGTKLEIK

SEQ ID NO: 76 - protein, 107 aa, synthetic construct
  REGION 1..107: note = VL
DIQMTQSPSSLSASVGDRVTITCKASQSVYHDVAWYQQKPGKAPKLLIYSASNRYTGVPSRFSGSGSGTDFTFTISSLQPEDIATYYCQHDYSSPYTFGQGTKLEIK

SEQ ID NO: 77 - protein, 107 aa, synthetic construct
  REGION 1..107: note = VL
DIQMTQSPSSLSASVGDRVTITCKASQSVYSDVAWYQQKPGKAPKLLIYSASNRYTGVPSRFSGSGSGTDFTFTISSLQPEDIATYYCQHDYSSPYTFGQGTKLEIK

SEQ ID NO: 78 - protein, 107 aa, synthetic construct
  REGION 1..107: note = VL
DIQMTQSPSSLSASVGDRVTITCKASQSVSNDLAWYQQKPGKAPKLLIYSASNRYTGVPSRFSGSGSGTDFTFTISSLQPEDIATYYCQHDYSSPYTFGQGTKLEIK

SEQ ID NO: 79 - protein, 107 aa, synthetic construct
  REGION 1..107: note = VL
DIQMTQSPSSLSASVGDRVTITCKASQSVSNDVAWYQQKPGKAPKLLIYRASNRYTGVPSRFSGSGSGTDFTFTISSLQPEDIATYYCQHDYSSPYTFGQGTKLEIK

SEQ ID NO: 80 - protein, 107 aa, synthetic construct
  REGION 1..107: note = VL
DIQMTQSPSSLSASVGDRVTITCKASQSVSNDVAWYQQKPGKAPKLLIYSASSRYTGVPSRFSGSGSGTDFTFTISSLQPEDIATYYCQHDYSSPYTFGQGTKLEIK

SEQ ID NO: 81 - protein, 107 aa, synthetic construct
  REGION 1..107: note = VL
DIQMTQSPSSLSASVGDRVTITCKASQSVSNDVAWYQQKPGKAPKLLIYSASRRYTGVPSRFSGSGSGTDFTFTISSLQPEDIATYYCQHDYSSPYTFGQGTKLEIK

SEQ ID NO: 82 - protein, 107 aa, synthetic construct
  REGION 1..107: note = VL
DIQMTQSPSSLSASVGDRVTITCKASQSVSNDVAWYQQKPGKAPKLLIYRASRRYTGVPSRFSGSGSGTDFTFTISSLQPEDIATYYCQHDYSSPYTFGQGTKLEIK

SEQ ID NO: 83 - protein, 107 aa, synthetic construct
  REGION 1..107: note = VL
DIQMTQSPSSLSASVGDRVTITCKASQSVSNDVAWYQQKPGKAPKLLIYRASSRYTGVPSRFSGSGSGTDFTFTISSLQPEDIATYYCQHDYSSPYTFGQGTKLEIK

SEQ ID NO: 84 - protein, 107 aa, synthetic construct
  REGION 1..107: note = VL
DIQMTQSPSSLSASVGDRVTITCKASQSVSNDVAWYQQKPGKAPKLLIYRASRRYPGVPSRFSGSGSGTDFTFTISSLQPEDIATYYCQHDYSSPYTFGQGTKLEIK

SEQ ID NO: 85 - protein, 107 aa, synthetic construct
  REGION 1..107: note = VL
DIQMTQSPSSLSASVGDRVTITCKASQSVYRDVAWYQQKPGKAPKLLIYRASNRYTGVPSRFSGSGSGTDFTFTISSLQPEDIATYYCQHDYSSPYTFGQGTKLEIK

SEQ ID NO: 86 - protein, 107 aa, synthetic construct
  REGION 1..107: note = VL
DIQMTQSPSSLSASVGDRVTITCKASQSVYRDVAWYQQKPGKAPKLLIYRASSRYTGVPSRFSGSGSGTDFTFTISSLQPEDIATYYCQHDYSSPYTFGQGTKLEIK

SEQ ID NO: 87 - protein, 107 aa, synthetic construct
  REGION 1..107: note = VL
DIQMTQSPSSLSASVGDRVTITCKASQSVYRDVAWYQQKPGKAPKLLIYSASNRYTGVPSRFSGSGSGTDFTFTISSLQPEDIATYYCQHDYSSPYTFGQGTKLEIK

SEQ ID NO: 88 - protein, 5 aa, synthetic construct
  REGION 1..5: note = H-CDR1
TYNMD

SEQ ID NO: 89 - protein, 17 aa, synthetic construct
  REGION 1..17: note = H-CDR2
TIYPGNGDTSYNQKFKG

SEQ ID NO: 90 - protein, 8 aa, synthetic construct
  REGION 1..8: note = H-CDR3
GDLYALDY

SEQ ID NO: 91 - protein, 11 aa, synthetic construct
  REGION 1..11: note = L-CDR1
KASQSVSNDVA

SEQ ID NO: 92 - protein, 7 aa, synthetic construct
  REGION 1..7: note = L-CDR2
SASNRYT

SEQ ID NO: 93 - protein, 9 aa, synthetic construct
  REGION 1..9: note = L-CDR3
QHDYSSPYT

SEQ ID NO: 94 - protein, 5 aa, synthetic construct
  REGION 1..5: note = H-CDR1
SFGMH

SEQ ID NO: 95 - protein, 10 aa, synthetic construct
  REGION 1..10: note = H-CDR2
YITSGSNTIY

SEQ ID NO: 96 - protein, 11 aa, synthetic construct
  REGION 1..11: note = H-CDR3
EYYSYDEGFAY

SEQ ID NO: 97 - protein, 12 aa, synthetic construct
  REGION 1..12: note = L-CDR1
SVSSSISSNYLH

SEQ ID NO: 98 - protein, 7 aa, synthetic construct
  REGION 1..7: note = L-CDR2
RTSNLAS

SEQ ID NO: 99 - protein, 9 aa, synthetic construct
  REGION 1..9: note = L-CDR3
QQGVDVPFT

SEQ ID NO: 100 - protein, 17 aa, synthetic construct
  REGION 1..17: note = H-CDR2
YITSGSNTIYYADTVKG

SEQ ID NO: 101 - protein, 17 aa, synthetic construct
  REGION 1..17: note = H-CDR2
YITPGSNTIYYADTVKG

SEQ ID NO: 102 - protein, 17 aa, synthetic construct
  REGION 1..17: note = H-CDR2
YITAGSNTIYYADTVKG

SEQ ID NO: 103 - protein, 17 aa, synthetic construct
  REGION 1..17: note = H-CDR2
YITPGSNTTYYADTVKG

SEQ ID NO: 104 - protein, 17 aa, synthetic construct
  REGION 1..17: note = H-CDR2
YITSGANTIYYADTVKG

SEQ ID NO: 105 - protein, 5 aa, synthetic construct
  REGION 1..5: note = H-CDR1
SFGMS

SEQ ID NO: 106 - protein, 17 aa, synthetic construct
  REGION 1..17: note = H-CDR2
YITPGSSTIYYADTVKG

SEQ ID NO: 107 - protein, 5 aa, synthetic construct
  REGION 1..5: note = H-CDR1
SYGMH

SEQ ID NO: 108 - protein, 17 aa, synthetic construct
  REGION 1..17: note = H-CDR2
SITPGSNTIYYADTVKG

SEQ ID NO: 109 - protein, 11 aa, synthetic construct
  REGION 1..11: note = H-CDR3
EYSSYDEGFAY

SEQ ID NO: 110 - protein, 17 aa, synthetic construct
  REGION 1..17: note = H-CDR2
VITPGSNTIYYADTVKG

SEQ ID NO: 111 - protein, 11 aa, synthetic construct
  REGION 1..11: note = H-CDR3
EYYSSDEGFAY

SEQ ID NO: 112 - protein, 11 aa, synthetic construct
  REGION 1..11: note = H-CDR3
EYYSYDEGPAY

SEQ ID NO: 113 - protein, 11 aa, synthetic construct
  REGION 1..11: note = H-CDR3
EYYSYDEGGAY

SEQ ID NO: 114 - protein, 11 aa, synthetic construct
  REGION 1..11: note = H-CDR3
EYYSYDEGFAS

SEQ ID NO: 115 - protein, 12 aa, synthetic construct
  REGION 1..12: note = L-CDR1
SVSSSIPSNYLH

SEQ ID NO: 116 - protein, 12 aa, synthetic construct
  REGION 1..12: note = L-CDR1
SVSSSISSKYLH

SEQ ID NO: 117 - protein, 12 aa, synthetic construct
  REGION 1..12: note = L-CDR1
SVSSLISSNYLH

SEQ ID NO: 118 - protein, 12 aa, synthetic construct
  REGION 1..12: note = L-CDR1
SVSDLISSNYLH

SEQ ID NO: 119 - protein, 12 aa, synthetic construct
  REGION 1..12: note = L-CDR1
SVSELLSTNYLH

SEQ ID NO: 120 - protein, 12 aa, synthetic construct
  REGION 1..12: note = L-CDR1
SVSSLIPSKYLH

SEQ ID NO: 121 - protein, 12 aa, synthetic construct
  REGION 1..12: note = L-CDR1
SVSDLIPSQYLH

SEQ ID NO: 122 - protein, 12 aa, synthetic construct
  REGION 1..12: note = L-CDR1
SVSDLIPSQYLS

SEQ ID NO: 123 - protein, 12 aa, synthetic construct
  REGION 1..12: note = L-CDR1
SVSDLIPSQYLA

SEQ ID NO: 124 - protein, 7 aa, synthetic construct
  REGION 1..7: note = L-CDR2
RASNLAS

SEQ ID NO: 125 - protein, 7 aa, synthetic construct
  REGION 1..7: note = L-CDR2
DASNLAS

SEQ ID NO: 126 - protein, 7 aa, synthetic construct
  REGION 1..7: note = L-CDR2
GASNLAS

SEQ ID NO: 127 - protein, 7 aa, synthetic construct
  REGION 1..7: note = L-CDR2
RTSNRAS

SEQ ID NO: 128 - protein, 199 aa, synthetic construct [sequence omitted]

SEQ ID NO: 129 - protein, 199 aa, synthetic construct
MNCVCRLVLVVLSLWPDRVVAPGPPAGSPRVSSDPRADLDSAVLLTRSLLADTRQLAAQMRDKFPADGDHSLDSLPTLAMSAGTLGSLQLPGVLTRLRVDLMSYLRHVQWLRRAGGPSLKTLEPELGALQARLERLLRRLQLLMSRLALPQAAPDQPVIPLGPPASAWGSIRAAHAILGGLHLTLDWAVRGLLLLKTRL

SEQ ID NO: 130 - protein, 8 aa, synthetic construct
  REGION 1..8: note = H-CDR3
GDLHFLDY

SEQ ID NO: 131 - protein, 8 aa, synthetic construct
  REGION 1..8: note = H-CDR3
GDLHYLDY

SEQ ID NO: 132 - protein, 5 aa, synthetic construct
  REGION 1..5: note = H-CDR1
TYDMD

SEQ ID NO: 133 - protein, 5 aa, synthetic construct
  REGION 1..5: note = H-CDR1
TYNID

SEQ ID NO: 134 - protein, 8 aa, synthetic construct
  REGION 1..8: note = H-CDR3
ADLHFLDY

SEQ ID NO: 135 - protein, 5 aa, synthetic construct
  REGION 1..5: note = H-CDR1
HYDMD

SEQ ID NO: 136 - protein, 5 aa, synthetic construct
  REGION 1..5: note = H-CDR1
TYDID

SEQ ID NO: 137 - protein, 5 aa, synthetic construct
  REGION 1..5: note = H-CDR1
TYDMH

SEQ ID NO: 138 - protein, 5 aa, synthetic construct
  REGION 1..5: note = H-CDR1
TYDMS

SEQ ID NO: 139 - protein, 5 aa, synthetic construct
  REGION 1..5: note = H-CDR1
HYNMD

SEQ ID NO: 140 - protein, 5 aa, synthetic construct
  REGION 1..5: note = H-CDR1
HYEMD

SEQ ID NO: 141 - protein, 5 aa, synthetic construct
  REGION 1..5: note = H-CDR1
HYQMD

SEQ ID NO: 142 - protein, 5 aa, synthetic construct
  REGION 1..5: note = H-CDR1
HYSMD

SEQ ID NO: 143 - protein, 17 aa, synthetic construct
  REGION 1..17: note = H-CDR2
TIYPGNADTSYNQKFKG

SEQ ID NO: 144 - protein, 17 aa, synthetic construct
  REGION 1..17: note = H-CDR2
TIYPGEGDTSYNQKFKG

SEQ ID NO: 145 - protein, 17 aa, synthetic construct
  REGION 1..17: note = H-CDR2
TIYPGQGDTSYNQKFKG

SEQ ID NO: 146 - protein, 11 aa, synthetic construct
  REGION 1..11: note = L-CDR1
KASKSVSNDVA

SEQ ID NO: 147 - protein, 11 aa, synthetic construct
  REGION 1..11: note = L-CDR1
KASYSVSNDVA

SEQ ID NO: 148 - protein, 11 aa, synthetic construct
  REGION 1..11: note = L-CDR1
KASHSVSNDVA

SEQ ID NO: 149 - protein, 11 aa, synthetic construct
  REGION 1..11: note = L-CDR1
KASQFVSNDVA

SEQ ID NO: 150 - protein, 11 aa, synthetic construct
  REGION 1..11: note = L-CDR1
KASQSVSNDIA

SEQ ID NO: 151 - protein, 11 aa, synthetic construct
  REGION 1..11: note = L-CDR1
KASQSVFHDVA

SEQ ID NO: 152 - protein, 11 aa, synthetic construct
  REGION 1..11: note = L-CDR1
KASQSVFRDVA

SEQ ID NO: 153 - protein, 11 aa, synthetic construct
  REGION 1..11: note = L-CDR1
KASQSVYHDVA

SEQ ID NO: 154 - protein, 11 aa, synthetic construct
  REGION 1..11: note = L-CDR1
KASQSVYSDVA

SEQ ID NO: 155 - protein, 11 aa, synthetic construct
  REGION 1..11: note = L-CDR1
KASQSVSNDLA

SEQ ID NO: 156 - protein, 7 aa, synthetic construct
  REGION 1..7: note = L-CDR2
RASNRYT

SEQ ID NO: 157 - protein, 7 aa, synthetic construct
  REGION 1..7: note = L-CDR2
SASSRYT

SEQ ID NO: 158 - protein, 7 aa, synthetic construct
  REGION 1..7: note = L-CDR2
SASRRYT

SEQ ID NO: 159 - protein, 7 aa, synthetic construct
  REGION 1..7: note = L-CDR2
RASRRYT

SEQ ID NO: 160 - protein, 7 aa, synthetic construct
  REGION 1..7: note = L-CDR2
RASSRYT

SEQ ID NO: 161 - protein, 7 aa, synthetic construct
  REGION 1..7: note = L-CDR2
RASRRYP

SEQ ID NO: 162 - protein, 11 aa, synthetic construct
  REGION 1..11: note = L-CDR1
KASQSVYRDVA